European Patent Application EP 4 245 864 A1, published September 20, 2023. Title: CHIP, PREPARATION METHOD THEREFOR, AND APPLICATION THEREOF. Applicant: GENEMIND BIOSCIENCES COMPANY LIMITED. The sequence listing filed with the application follows.

SEQUENCE LISTING (3 sequences)

SEQ ID NO: 1 - DNA, 61 bp, Artificial Sequence
  misc_feature (1)..(61): Sequence of adapter
tttttttttttccttgatacctgcgaccatccagttccactcagatgtgtataagagacag

SEQ ID NO: 2 - DNA, 30 bp, Artificial Sequence
  misc_feature (1)..(30): Sequence of adapter
ttttttttttaatgatacggcgaccaccga

SEQ ID NO: 3 - DNA, 31 bp, Artificial Sequence
  misc_feature (1)..(31): Sequence of adapter
ttttttttttcaagcagaagacggcatacga